European Patent Application EP 4 814 018 A2, published September 30, 2026. Title: ANTI-TRANSFERRIN RECEPTOR ANTIBODIES WITH TAILORED AFFINITY. Applicant: F. Hoffmann-La Roche AG. The sequence listing filed with the application follows.

SEQUENCE LISTING (97 sequences)

SEQ ID NO: 1 - protein, 122 aa, Oryctolagus cuniculus
QSMEESGGRLVTPGTPLTLTCTVSGFSLSSYAMSWVRQAPGKGLEWIGYIWSGGSTDYASWAKGRFTISKTSTTVDLKITSPTTEDTATYFCARRYGTSYPDYGDANGFDPWGPGTLVTVSS

SEQ ID NO: 2 - protein, 122 aa, synthetic construct; identical to SEQ ID NO: 1
  REGION 1..122: note = anti-TfR mAb 567 VH (=humanized 299 VH_basic)

SEQ ID NO: 3 - protein, 124 aa, synthetic construct
  REGION 1..124: note = 299-001 VH humanization variant
VQLVETGGGLIQPGGSLRLSCAASGFSLSSYAMSWVRQAPGKGLEWVGYIWSGGSTDYADSVKGRFTISRDNSKNTLYLQMNSLRAEDTAVYYCARRYGTSYPDYGDANGFDPWGQGTLVTVSS

SEQ ID NO: 4 - protein, 125 aa, synthetic construct
  REGION 1..125: note = 299-002 VH humanization variant
EVQLVETGGGLIQPGGSLRLSCAASGFSLSSYAMSWVRQAPGKGLEWVGYIWSGGSTDYADSVKGRFTISRDNSKNTLYLQMNSLRAEDTAVYYCARRYGTSYPDYGDANGFDPWGQGTLVTVSS

SEQ ID NO: 5 - protein, 124 aa, synthetic construct
  REGION 1..124: note = 299-005 VH humanization variant
QSMEETGGGLIQPGGSLRLSCAASGFSLSSYAMSWVRQAPGKGLEWVGYIWSGGSTDYADSVKGRFTISRDNSKNTLYLQMNSLRAEDTAVYYCARRYGTSYPDYGDANGFDPWGPGTLVTVSS

SEQ ID NO: 6 - protein, 124 aa, synthetic construct
  REGION 1..124: note = 299-006 VH humanization variant
QQLVETGGGLIQPGGSLRLSCAASGFSLSSYAMSWVRQAPGKGLEWIGYIWSGGSTDYADSVKGRFTISRDNSKNTLYLQMNSLRAEDTAVYYCARRYGTSYPDYGDANGFDPWGQGTLVTVSS

SEQ ID NO: 7 - protein, 124 aa, synthetic construct
  REGION 1..124: note = 299-007 VH humanization variant_DANG
QQLVETGGGLIQPGGSLRLSCAASGFSLSSYAMSWVRQAPGKGLEWIGYIWSGGSTDYASWAKGRFTISRDNSKNTLYLQMNSLRAEDTAVYYCARRYGTSYPDYGDANGFDPWGQGTLVTVSS

SEQ ID NO: 8 - protein, 122 aa, synthetic construct
  REGION 1..122: note = 299-008 VH humanization variant
QQLVETGGGLIQPGGSLRLSCAASGFSLSSYAMSWVRQAPGKGLEWIGYIWSGGSTDYASWAKGRFTISKTSTTLYLQMNSLRAEDTAVYYCARRYGTSYPDYGDANGFDPWGQGTLVTVSS

SEQ ID NO: 9 - protein, 124 aa, synthetic construct
  REGION 1..124: note = 299-009 VH humanization variant_DANG
QQLLESGGGLVQPGGSLRLSCAASGFTFSSYAMSWVRQAPGKGLEWVGYIWSGGSTDYADSVKGRFTISRDNSKNTLYLQMNSLRAEDTAVYYCAKRYGTSYPDYGDANGFDPWGQGTLVTVSS

SEQ ID NO: 10 - protein, 124 aa, synthetic construct
  REGION 1..124: note = 299-009 VH humanization variant_DASG
QQLLESGGGLVQPGGSLRLSCAASGFTFSSYAMSWVRQAPGKGLEWVGYIWSGGSTDYADSVKGRFTISRDNSKNTLYLQMNSLRAEDTAVYYCAKRYGTSYPDYGDASGFDPWGQGTLVTVSS

SEQ ID NO: 11 - protein, 124 aa, synthetic construct
  REGION 1..124: note = 299-009 VH humanization variant_DAQG
QQLLESGGGLVQPGGSLRLSCAASGFTFSSYAMSWVRQAPGKGLEWVGYIWSGGSTDYADSVKGRFTISRDNSKNTLYLQMNSLRAEDTAVYYCAKRYGTSYPDYGDAQGFDPWGQGTLVTVSS

SEQ ID NO: 12 - protein, 124 aa, synthetic construct
  REGION 1..124: note = 299-011 VH humanization variant
QQLLESGGGLVQPGGSLRLSCAASGFSLSSYAMSWVRQAPGKGLEWVGYIWSGGSTDYADSVKGRFTISRDNSKNTLYLQMNSLRAEDTAVYYCARRYGTSYPDYGDANGFDPWGQGTLVTVSS

SEQ ID NO: 13 - protein, 125 aa, synthetic construct
  REGION 1..125: note = 299-012 VH humanization variant
QVQLQESGPGLVKPSETLSLTCTVSGFSLSSYAMSWIRQPPGKGLEWIGYIWSGGSTDYNPSLKSRVTISVDTSKNQFSLKLSSVTAADTAVYYCARRYGTSYPDYGDANGFDPWGQGTLVTVSS

SEQ ID NO: 14 - protein, 125 aa, synthetic construct
  REGION 1..125: note = 299-013 VH humanization variant
QVQLQESGPGLVKPSETLSLTCTVSGFSLSSYAMSWIRQPPGKGLEWIGYIWSGGSTDYNPSLKSRVTISVDTSKNQVSLKLSSVTAADTAVYYCARRYGTSYPDYGDANGFDPWGQGTLVTVSS

SEQ ID NO: 15 - protein, 124 aa, synthetic construct
  REGION 1..124: note = 299-015 VH humanization variant
QQLQESGPGLVKPSETLSLTCTVSGFSLSSYAMSWVRQPPGKGLEWIGYIWSGGSTDYNPSLKSRVTISVDTSKNQVSLKLSSVTAADTAVYYCARRYGTSYPDYGDANGFDPWGQGTLVTVSS

SEQ ID NO: 16 - protein, 124 aa, synthetic construct
  REGION 1..124: note = 299-016 VH humanization variant
QQLQESGPGLVKPSETLSLTCTVSGFSLSSYAMSWVRQPPGKGLEWIGYIWSGGSTDYNPSLKSRVTISVDTSKNQVSLKLSSVTAADTAVYYCARRYGTSYPDYGDANGFDPWGPGTLVTVSS

SEQ ID NO: 17 - protein, 124 aa, synthetic construct
  REGION 1..124: note = 299-017 VH humanization variant
QQLQESGPGLVKPSETLSLTCTVSGFSLSSYAMSWVRQPPGKGLEWIGYIWSGGSTDYNPSLKSRVTISKDTSKNQVSLKLSSVTAADTAVYYCARRYGTSYPDYGDANGFDPWGPGTLVTVSS

SEQ ID NO: 18 - protein, 125 aa, synthetic construct
  REGION 1..125: note = 299-018 VH humanization variant
QVQLQESGPGLVKPSQTLSLTCTVSGFSLSSYAMSWIRQHPGKGLEWIGYIWSGGSTDYAPSLKSRVTISVDTSKNQFSLKLSSVTAADTAVYYCARRYGTSYPDYGDANGFDPWGQGTLVTVSS

SEQ ID NO: 19 - protein, 124 aa, synthetic construct
  REGION 1..124: note = 299-019 VH humanization variant
QSMQESGPGLVKPSQTLSLTCTVSGFSLSSYAMSWIRQHPGKGLEWIGYIWSGGSTDYAPSLKSRVTISVDTSKNQFSLKLSSVTAADTAVYYCARRYGTSYPDYGDANGFDPWGQGTLVTVSS

SEQ ID NO: 20 - protein, 124 aa, synthetic construct
  REGION 1..124: note = 299-020 VH humanization variant
QSMQESGPGLVKPSQTLSLTCTVSGFSLSSYAMSWIRQHPGKGLEWIGYIWSGGSTDYAPSLKSRVTISVDTSKNQVSLKLSSVTAADTAVYYCARRYGTSYPDYGDANGFDPWGQGTLVTVSS

SEQ ID NO: 21 - protein, 124 aa, synthetic construct
  REGION 1..124: note = 299-021 VH humanization variant
QSMQESGPGLVKPSQTLSLTCTVSGFSLSSYAMSWIRQHPGKGLEWIGYIWSGGSTDYASWAKSRVTISVDTSKNQVSLKLSSVTAADTAVYYCARRYGTSYPDYGDANGFDPWGQGTLVTVSS

SEQ ID NO: 22 - protein, 124 aa, synthetic construct
  REGION 1..124: note = 299-022 VH humanization variant
QSMQESGPGLVKPSQTLSLTCTVSGFSLSSYAMSWVRQHPGKGLEWIGYIWSGGSTDYASWAKSRVTISVDTSKNQVSLKLSSVTAADTAVYYCARRYGTSYPDYGDANGFDPWGQGTLVTVSS

SEQ ID NO: 23 - protein, 122 aa, synthetic construct
  REGION 1..122: note = 299-023 VH humanization variant_DANG
QSMQESGPGLVKPSQTLSLTCTVSGFSLSSYAMSWIRQHPGKGLEWIGYIWSGGSTDYASWAKSRVTISKTSTTVSLKLSSVTAADTAVYYCARRYGTSYPDYGDANGFDPWGQGTLVTVSS

SEQ ID NO: 24 - protein, 122 aa, synthetic construct
  REGION 1..122: note = 299-023 VH humanization variant_DASG
QSMQESGPGLVKPSQTLSLTCTVSGFSLSSYAMSWIRQHPGKGLEWIGYIWSGGSTDYASWAKSRVTISKTSTTVSLKLSSVTAADTAVYYCARRYGTSYPDYGDASGFDPWGQGTLVTVSS

SEQ ID NO: 25 - protein, 122 aa, synthetic construct
  REGION 1..122: note = 299-023 VH humanization variant_DAQG
QSMQESGPGLVKPSQTLSLTCTVSGFSLSSYAMSWIRQHPGKGLEWIGYIWSGGSTDYASWAKSRVTISKTSTTVSLKLSSVTAADTAVYYCARRYGTSYPDYGDAQGFDPWGQGTLVTVSS

SEQ ID NO: 26 - protein, 110 aa, Oryctolagus cuniculus
AYDMTQTPASVEVAVGGTVTIKCQASQSISSYLSWYQQKPGQRPKLLIYRASTLASGVSSRFKGSGSGTQFTLTISGVECADAATYYCQQCYSSSNVDNTFGGGTEVVVK

SEQ ID NO: 27 - protein, 110 aa, synthetic construct
  REGION 1..110: note = anti-TfR mAb 567 VL (=humanized 299 VL_basic)
AYDMTQTPASVEVAVGGTVTIKCQASQSISSYLSWYQQKPGQRPKLLIYRASTLASGVSSRFKGSGSGTQFTLTISGVESADAATYYCQQSYSSSNVDNTFGGGTEVVVK

SEQ ID NO: 28 - protein, 110 aa, synthetic construct
  REGION 1..110: note = 567 VL humanization variant_PNYA
AYDMTQTPASVEVAVGGTVTIKCQASQSISSYLSWYQQKPGQRPKLLIYRASTLASGVSSRFKGSGSGTQFTLTISGVEPADAATYYCQQNYASSNVDNTFGGGTEVVVK

SEQ ID NO: 29 - protein, 110 aa, synthetic construct
  REGION 1..110: note = 299-001 VL humanization variant
DIQMTQSPSSLSASVGDRVTITCRASQSISSYLNWYQQKPGKAPKLLIYRASSLQSGVPSRFSGSGSGTDFTLTISSLQPEDFATYYCQQSYSSSNVDNTFGGGTKVEIK

SEQ ID NO: 30 - protein, 110 aa, synthetic construct
  REGION 1..110: note = 299-002 VL humanization variant_SYS
DIQMTQSPSSLSASVGDRVTITCRASQSISSYLNWYQQKPGKAPKLLIYRASTLASGVPSRFSGSGSGTDFTLTISSLQPEDFATYYCQQSYSSSNVDNTFGGGTKVEIK

SEQ ID NO: 31 - protein, 110 aa, synthetic construct
  REGION 1..110: note = 299-003 VL humanization variant
AYQMTQSPSSLSASVGDRVTITCRASQSISSYLNWYQQKPGKAPKLLIYRASTLASGVPSRFSGSGSGTDFTLTISSLQPEDFATYYCQQSYSSSNVDNTFGGGTKVEIK

SEQ ID NO: 32 - protein, 110 aa, synthetic construct
  REGION 1..110: note = 299-004 VL humanization variant
AYQMTQSPSSLSASVGDRVTITCRASQSISSYLSWYQQKPGKAPKLLIYRASTLASGVPSRFSGSGSGTDFTLTISSLQPEDFATYYCQQSYSSSNVDNTFGGGTKVEIK

SEQ ID NO: 33 - protein, 110 aa, synthetic construct
  REGION 1..110: note = 299-005 VL humanization variant
DIQMTQSPSSLSASVGDRVTITCRASQSISSYLSWYQQKPGKAPKLLIYRASTLASGVPSRFSGSGSGTDFTLTISSLQPEDFATYYCQQSYSSSNVDNTFGGGTKVEIK

SEQ ID NO: 34 - protein, 110 aa, synthetic construct
  REGION 1..110: note = 299-006 VL humanization variant_SYS
AIQLTQSPSSLSASVGDRVTITCRASQSISSYLSWYQQKPGKAPKLLIYRASTLASGVPSRFSGSGSGTDFTLTISSLQPEDFATYYCQQSYSSSNVDNTFGGGTKVEIK

SEQ ID NO: 35 - protein, 110 aa, synthetic construct
  REGION 1..110: note = 299-007 VL humanization variant
AIQLTQSPSSLSASVGDRVTITCRASQSISSYLAWYQQKPGKAPKLLIYRASTLASGVPSRFSGSGSGTDFTLTISSLQPEDFATYYCQQSYSSSNVDNTFGGGTKVEIK

SEQ ID NO: 36 - protein, 110 aa, synthetic construct
  REGION 1..110: note = 299-008 VL humanization variant
AYQLTQSPSSLSASVGDRVTITCRASQSISSYLSWYQQKPGKAPKLLIYRASTLASGVPSRFSGSGSGTDFTLTISSLQPEDFATYYCQQSYSSSNVDNTFGGGTKVEIK

SEQ ID NO: 37 - protein, 110 aa, synthetic construct
  REGION 1..110: note = 299-009 VL humanization variant_NYA
AIQLTQSPSSLSASVGDRVTITCRASQSISSYLAWYQQKPGKAPKLLIYRASTLASGVPSRFSGSGSGTDFTLTISSLQPEDFATYYCQQNYASSNVDNTFGGGTKVEIK

SEQ ID NO: 38 - protein, 110 aa, synthetic construct
  REGION 1..110: note = 299-009 VL humanization variant_SYA
AIQLTQSPSSLSASVGDRVTITCRASQSISSYLAWYQQKPGKAPKLLIYRASTLASGVPSRFSGSGSGTDFTLTISSLQPEDFATYYCQQSYASSNVDNTFGGGTKVEIK

SEQ ID NO: 39 - protein, 110 aa, synthetic construct
  REGION 1..110: note = 299-009 VL humanization variant_NYS
AIQLTQSPSSLSASVGDRVTITCRASQSISSYLAWYQQKPGKAPKLLIYRASTLASGVPSRFSGSGSGTDFTLTISSLQPEDFATYYCQQNYSSSNVDNTFGGGTKVEIK

SEQ ID NO: 40 - protein, 110 aa, synthetic construct
  REGION 1..110: note = 299-009 VL humanization variant_GYS
AIQLTQSPSSLSASVGDRVTITCRASQSISSYLAWYQQKPGKAPKLLIYRASTLASGVPSRFSGSGSGTDFTLTISSLQPEDFATYYCQQGYSSSNVDNTFGGGTKVEIK

SEQ ID NO: 41 - protein, 110 aa, synthetic construct
  REGION 1..110: note = 299-009 VL humanization variant_CYS
AIQLTQSPSSLSASVGDRVTITCRASQSISSYLAWYQQKPGKAPKLLIYRASTLASGVPSRFSGSGSGTDFTLTISSLQPEDFATYYCQQCYSSSNVDNTFGGGTKVEIK

SEQ ID NO: 42 - protein, 110 aa, synthetic construct
  REGION 1..110: note = 299-010 VL humanization variant
DIQMTQSPSSLSASVGDRVTITCRASQSISSYLSWYQQKPGKAPKLLIYRASTLASGVPSRFSGSRSGTDFTLTISSLQPEDFATYYCQQSYSSSNVDNTFGGGTKVEIK

SEQ ID NO: 43 - protein, 110 aa, synthetic construct
  REGION 1..110: note = 299-012 VL humanization variant_HYS
DIQMTQSPSSLSASVGDRVTITCRASQSISSYLAWYQQKPGKAPKLLIYRASTLASGVPSRFSGSRSGTDFTLTISSLQPEDFATYYCQQHYSSSNVDNTFGGGTKVEIK

SEQ ID NO: 44 - protein, 110 aa, synthetic construct
  REGION 1..110: note = 299-014 VL humanization variant
DIVMTQSPDSLAVSLGERATINCKSSQSISSYLSWYQQKPGQRPKLLIYRASTLASGVPDRFSGSGSGTDFTLTISSLQAEDVAVYYCQQSYSSSNVDNTFGGGTKVEIK

SEQ ID NO: 45 - protein, 110 aa, synthetic construct
  REGION 1..110: note = 299-015 VL humanization variant_AYS
DIVMTQSPDSLAVSLGERATINCKSSQSISSYLIWYQQKPGQPPKLLIYRASTLASGVPDRFSGSGSGTDFTLTISSLQAEDVAVYYCQQAYSSSNVDNTFGGGTKVEIK

SEQ ID NO: 46 - protein, 110 aa, synthetic construct
  REGION 1..110: note = 299-017 VL humanization variant_TYS
AIQLTQSPSSLSASVGDRVTITCRASQSISSYLAWYQQKPGKAPKLLIYRASTLASGVPSRFSGSGSGTDFTLTISSLQPEDFATYYCQQTYSSSNVDNTFGGGTKVEIK

SEQ ID NO: 47 - protein, 119 aa, Mus musculus
EVQLQQSGAVLVKPGASVKLSCPASGFNIKDTYIHWVIQRPEQGLEWIGRIDPANGDTKCDPKFQVKATITADTSSNTAYLQLSSLTSEDTAVYFCVRDYLYPYYFDFWGQGTTLTVSS

SEQ ID NO: 48 - protein, 119 aa, synthetic construct
  REGION 1..119: note = 494 VH variant D52A
EVQLQQSGAVLVKPGASVKLSCPASGFNIKDTYIHWVIQRPEQGLEWIGRIAPANGDTKSDPKFQVKATITADTSSNTAYLQLSSLTSEDTAVYFCVRDYLYPYYFDFWGQGTTLTVSS

SEQ ID NO: 49 - protein, 119 aa, synthetic construct
  REGION 1..119: note = 494 VH variant D52L
EVQLQQSGAVLVKPGASVKLSCPASGFNIKDTYIHWVIQRPEQGLEWIGRILPANGDTKSDPKFQVKATITADTSSNTAYLQLSSLTSEDTAVYFCVRDYLYPYYFDFWGQGTTLTVSS

SEQ ID NO: 50 - protein, 119 aa, synthetic construct
  REGION 1..119: note = 494 VH variant D31G
EVQLQQSGAVLVKPGASVKLSCPASGFNIKGTYIHWVIQRPEQGLEWIGRIDPANGDTKSDPKFQVKATITADTSSNTAYLQLSSLTSEDTAVYFCVRDYLYPYYFDFWGQGTTLTVSS

SEQ ID NO: 51 - protein, 119 aa, synthetic construct
  REGION 1..119: note = 494 VH variant L101A
EVQLQQSGAVLVKPGASVKLSCPASGFNIKDTYIHWVIQRPEQGLEWIGRIDPANGDTKSDPKFQVKATITADTSSNTAYLQLSSLTSEDTAVYFCVRDYAYPYYFDFWGQGTTLTVSS

SEQ ID NO: 52 - protein, 119 aa, synthetic construct
  REGION 1..119: note = 494-001 VH humanization variant
QVQLVQSGAEVKKPGASVKVSCKASGFNIKDTYIHWVIQAPGQGLEWMGRIDPANGDTKSDPKFQVRVTITADTSTSTVYMELSSLRSEDTAVYYCVRDYLYPYYFDFWGQGTTVTVSS

SEQ ID NO: 53 - protein, 119 aa, synthetic construct
  REGION 1..119: note = 494-002 VH humanization variant
QVQLVQSGAEVKKPGASVKVSCKASGFNIKDTYIHWVIQAPGQGLEWMGRIDPANGDTKSAPKFQVRVTITADTSTSTVYMELSSLRSEDTAVYYCVRDYLYPYYFDFWGQGTTVTVSS

SEQ ID NO: 54 - protein, 119 aa, synthetic construct
  REGION 1..119: note = 494-003 VH humanization variant
QVQLVQSGAEVKKPGASVKVSCKASGFNIKDTYIHWVIQAPGQGLEWMGRIDPANGDTKSDPKFQGRVTITADTSTSTVYMELSSLRSEDTAVYYCVRDYLYPYYFDFWGQGTTVTVSS

SEQ ID NO: 55 - protein, 119 aa, synthetic construct
  REGION 1..119: note = 494-004 VH humanization variant
QVQLVQSGAEVKKPGSSVKVSCKASGFNIKDTYIHWVIQAPGQGLEWMGRIDPANGDTKSDPKFQGRVTITADESTSTAYMELSSLRSEDTAVYYCVRDYLYPYYFDFWGQGTTVTVSS

SEQ ID NO: 56 - protein, 119 aa, synthetic construct
  REGION 1..119: note = 494-005 VH humanization variant
QVQLVQSGAEVKKPGSSVKVSCKASGFNIKDTYIHWVIQRPGQGLEWMGRIDPANGDTKSDPKFQGRVTITADESTSTAYMELSSLRSEDTAVYYCVRDYLYPYYFDFWGQGTTVTVSS

SEQ ID NO: 57 - protein, 119 aa, synthetic construct
  REGION 1..119: note = 494-006 VH humanization variant
QVQLQESGPGLVKPSETLSLTCTVSGFNIKDTYIHWVIQRPGKGLEWIGRIDPANGDTKSDPSLQSRVTISADTSKNQASLKLSSVTAADTAVYYCVRDYLYPYYFDFWGQGTTVTVSS

SEQ ID NO: 58 - protein, 119 aa, synthetic construct
  REGION 1..119: note = 494-007 VH humanization variant
EVQLVESGGGLVQPGGSLRLSCAASGFNIKDTYIHWVIQAPGKGLEWVGRIDPANGDTKSDPSVQVRATISADTSKNTAYLQMNSLRAEDTAVYYCVRDYLYPYYFDFWGQGTTVTVSS

SEQ ID NO: 59 - protein, 107 aa, Mus musculus
KIVMTQSPKSMSMSVGERVTLNCRASESVDTYVSWYQQKPEQSPELLIYGASNRYTGVPDRFTGSGSATDFTLTISSVQAEDLADYYCGQTYNYPLTFGAGTKLELK

SEQ ID NO: 60 - protein, 107 aa, synthetic construct
  REGION 1..107: note = 494-001 VL humanization variant
KIQMTQSPSSLSASVGDRVTITCRASESVDTYVSWYQQKPGKAPKLLIYGASNRYTGVPSRFSGSGSGTDFTLTISSLQPEDFADYYCGQTYNYPLTFGQGTKLEIK

SEQ ID NO: 61 - protein, 107 aa, synthetic construct
  REGION 1..107: note = 494-002 VL humanization variant
KIVLTQSPGTLSLSPGERATLSCRASESVDTYVSWYQQKPGQAPRLLIYGASNRYTGVPDRFSGSGSGTDFTLTISRLEPEDFADYYCGQTYNYPLTFGQGTKLEIK

SEQ ID NO: 62 - protein, 107 aa, synthetic construct
  REGION 1..107: note = 494-003 VL humanization variant
EIVLTQSPGTLSLSPGERATLSCRASESVDTYVSWYQQKPGQAPRLLIYGASNRYTGVPDRFSGSGSGTDFTLTISRLEPEDFADYYCGQTYNYPLTFGQGTKLEIK

SEQ ID NO: 63 - protein, 107 aa, synthetic construct
  REGION 1..107: note = 494-004 VL humanization variant
KIVLTQSPGTLSLSPGERATLSCRASESVDTYVSWYQQKPGQAPRLLIYGASNRYTGIPDRFSGSGSGTDFTLTISRLEPEDFADYYCGQTYNYPLTFGQGTKLEIK

SEQ ID NO: 64 - protein, 118 aa, Mus musculus
QVQLVQSGAEVKKPGASVKVSCKASGYTFTGYTMNWVRQAPGQGLEWMGRINPHNGGTDYAQKFQGRVTMTRDTSISTAYMELSRLRSDDTAVYYCARGYYYYSLDYWGQGTLVTVSS

SEQ ID NO: 65 - protein, 106 aa, Mus musculus
DIQMTQSPSSLSASVGDRVTITCRASSSIRYIHWYQQKPGKAPKRLIYDTSNLASGVPSRFSGSGSGTEFTLTISSLQPEDFATYYCHQRNSYPWTFGQGTRLEIK

SEQ ID NO: 66 - protein, 7 aa, Oryctolagus cuniculus
GFSLSSY

SEQ ID NO: 67 - protein, 5 aa, Oryctolagus cuniculus
SYAMS

SEQ ID NO: 68 - protein, 5 aa, Oryctolagus cuniculus
WSGGS

SEQ ID NO: 69 - protein, 16 aa, Oryctolagus cuniculus
YIWSGGSTDYASWAKG

SEQ ID NO: 70 - protein, 16 aa, synthetic construct
  REGION 1..16: note = 299-000 HVR-H2 Kabat G65S
YIWSGGSTDYASWAKS

SEQ ID NO: 71 - protein, 17 aa, Oryctolagus cuniculus
RYGTSYPDYGDANGFDP

SEQ ID NO: 72 - protein, 17 aa, synthetic construct
  REGION 1..17: note = 299-000 HVR-H3 DASG
RYGTSYPDYGDASGFDP

SEQ ID NO: 73 - protein, 17 aa, synthetic construct
  REGION 1..17: note = 299-000 HVR-H3 DAQG
RYGTSYPDYGDAQGFDP

SEQ ID NO: 74 - protein, 11 aa, Oryctolagus cuniculus
QASQSISSYLS

SEQ ID NO: 75 - protein, 11 aa, synthetic construct
  REGION 1..11: note = 299-000 HVR-L1 RAA
RASQSISSYLA

SEQ ID NO: 76 - protein, 7 aa, Oryctolagus cuniculus
RASTLAS

SEQ ID NO: 77 - protein, 12 aa, Oryctolagus cuniculus
QQCYSSSNVDNT

SEQ ID NO: 78 - protein, 12 aa, synthetic construct
  REGION 1..12: note = 299-000 HVR-L3 NYA
QQNYASSNVDNT

SEQ ID NO: 79 - protein, 119 aa, synthetic construct
  REGION 1..119: note = anti-CD20 antibody VH
QVQLVQSGAEVKKPGSSVKVSCKASGYAFSYSWINWVRQAPGQGLEWMGRIFPGDGDTDYNGKFKGRVTITADKSTSTAYMELSSLRSEDTAVYYCARNVFDGYWLVYWGQGTLVTVSS

SEQ ID NO: 80 - protein, 112 aa, synthetic construct
  REGION 1..112: note = anti-CD20 antibody VL
DIVMTQTPLSLPVTPGEPASISCRSSKSLLHSNGITYLYWYLQKPGQSPQLLIYQMSNLVSGVPDRFSGSGSGTDFTLKISRVEAEDVGVYYCAQNLELPYTFGGGTKVEIK

SEQ ID NO: 81 - protein, 126 aa, Homo sapiens [sequence omitted]

SEQ ID NO: 82 - protein, 108 aa, Homo sapiens [sequence omitted]

SEQ ID NO: 83 - protein, 116 aa, synthetic construct
  REGION 1..116: note = humanized anti-alpha synuclein acntibody 9E4 VH
EVQLVESGGGLVQPGGSLRLSCAASGFTFSNYGMSWVRQAPGKGLEWVASISSGGGSTYYPDNVKGRFTISRDDAKNSLYLQMNSLRAEDTAVYYCARGGAGIDYWGQGTLVTVSS

SEQ ID NO: 84 - protein, 113 aa, synthetic construct
  REGION 1..113: note = humanized anti-alpha synuclein acntibody 9E4 VL
DIQMTQSPSSLSASVGDRVTITCKSIQTLLYSSNQKNYLAWFQQKPGKAPKLLIYWASIRKSGVPSRFSGSGSGTDFTLTISSLQPEDLATYYCQQYYSYPLTFGGGTKLEIK

SEQ ID NO: 85 - protein, 115 aa, Mus musculus
QVQLQQSGAELAKPGTSVQMSCKASGYTFTNYWMNWIKARPGQGLEWIGATNPNNGYTDYNQRFKDKAILTADKSSNTAYMHLSSLTSEDSAVYFCASGGHLAYWGQGTVVTVSA

SEQ ID NO: 86 - protein, 112 aa, Mus musculus
DVVMTQIPLYLSVSPGDQASISCRSSQSLFHSKGNTYLHWYLQKPGQSPKLLINRVSNRFSGVPDRFSGSGSGTDFTLKISGVEAEDLGVYFCSQSAHVPWTFGGGTKLEIR

SEQ ID NO: 87 - protein, 115 aa, Mus musculus
VQLQQSGPELVKPGTSVKISCKASGYSFTSYYIHWVKQSPGQGLEWIGWIYPGSGNTKYSEKFKGKATLTADTSSSTAYMQLSSLTSEDSAVYFCARDGCYGFAYWGQGTLVTVS

SEQ ID NO: 88 - protein, 111 aa, Mus musculus
DIVLTQSPASLAVSLGQRATISCKASQSVDYDGDSYMNWYQQKPGQPPKFLICAASNLESGIPARFSGSGSGTDFTLNIHPVEEEDAATYYCQQSNEDPFTFGSGTKLEIK

SEQ ID NO: 89 - protein, 115 aa, Oryctolagus cuniculus
QSVEESGGRLVTPGTPLTLTCTVSGFSINSYAMIWVRQAPGEGLEWIGVIYPSGNTYYANWAKGRFTVSRTSTTVDLKITSPTTEDTATYFCARRDGTDKTFNIWGPGTLVTVSL

SEQ ID NO: 90 - protein, 112 aa, Oryctolagus cuniculus
QVLTQTPSPVSAAVGGTVTINCQASQNVYGDNYLAWYQQKPGQPPKLLIYEASKLASGVPPRFSGSGSGTQFTLTISDVQCDDAATYYCQGEFLCTTSDCFTFGGGTGVVVR

SEQ ID NO: 91 - protein, 119 aa, Oryctolagus cuniculus
QSVEESGGRLVTPGTPLTLTCTVSGIDLSRYAMSWVRQAPGKGLEWIGVINSSGATYYASWAKGRFTISETSTTVELKITSPTTEDTATYFCARWTYDDYGDFQGFNIWGPGTLVTVSL

SEQ ID NO: 92 - protein, 111 aa, Oryctolagus cuniculus
AVLTQTPSPVSAAVGGTVTISCQSSQSVYNNNDLAWYQQKPGQPPKLLIYRASKLASGVPSRFKGSGSGTQFTLTISGVQCDDAATYYCLGGYDDDADMGAFGGGTEVVVK

SEQ ID NO: 93 - protein, 111 aa, synthetic construct
  REGION 1..111: note = heavy chain variable domain
QSLEESGGRLVTPGTPLTLTCTVSGIDLSRDTMIWVRQAPGEGLEWIGSIYTDSGNTWYASWVKGRFTISKTSSTTVDLRITSPTTEDTATYFCARNFSVWGPGTLVTVSL

SEQ ID NO: 94 - protein, 112 aa, synthetic construct
  REGION 1..112: note = light chain variable domain
QVLTQTPSPVSAAVGGTVTINCQASQSVYNSDRLAWFQQMRGQPPKLLIYDVSKLASGVPSRFSGSGSGTQFTLTISDVQCDDAATYYCLGGYDCSSAECNVFGGGTEVVVK

SEQ ID NO: 95 - protein, 20 aa, synthetic construct
  REGION 1..20: note = peptidic linker
GGGGSGGGGSGGGGSGGGGS

SEQ ID NO: 96 - protein, 32 aa, synthetic construct
  REGION 1..32: note = peptidic linker
GGGGSGGGGSGGGGSGGGGSGGGGSGGGGSGG

SEQ ID NO: 97 - protein, 536 aa, Homo sapiens
MEFSSPSREECPKPLSRVSIMAGSLTGLLLLQAVSWASGARPCIPKSFGYSSVVCVCNATYCDSFDPPTFPALGTFSRYESTRSGRRMELSMGPIQANHTGTGLLLTLQPEQKFQKVKGFGGAMTDAAALNILALSPPAQNLLLKSYFSEEGIGYNIIRVPMASCDFSIRTYTYADTPDDFQLHNFSLPEEDTKLKIPLIHRALQLAQRPVSLLASPWTSPTWLKTNGAVNGKGSLKGQPGDIYHQTWARYFVKFLDAYAEHKLQFWAVTAENEPSAGLLSGYPFQCLGFTPEHQRDFIARDLGPTLANSTHHNVRLLMLDDQRLLLPHWAKVVLTDPEAAKYVHGIAVHWYLDFLAPAKATLGETHRLFPNTMLFASEACVGSKFWEQSVRLGSWDRGMQYSHSIITNLLYHVVGWTDWNLALNPEGGPNWVRNFVDSPIIVDITKDTFYKQPMFYHLGHFSKFIPEGSQRVGLVASQKNDLDAVALMHPDGSAVVVVLNRSSKDVPLTIKDPAVGFLETISPGYSIHTYLWRRQ